European Patent Application EP 4 748 928 A1, published May 27, 2026. Title: 신규한 제아랄레논 분해 효소 및 그의 용도. Applicant: 씨제이제일제당 주식회사. The sequence listing filed with the application follows.

SEQUENCE LISTING (8 sequences)

SEQ ID NO: 1 - protein, 316 aa, Sphingomonas sp.
MTSETGAPHPAHRNIFVSHSFPEQQVDLGEVTLNYVEAGDAGKPALLLVPEQTGSWWSYEPSIAMLAENFHVFAVDMRGQGRSDWTPRRYSLDNFGNDLVRFIALVIKRPTIVAGNSSGGVLAAWLSAYAMPGQIRGALCEDAPFFASELTPAYGHPIRQAAGPAFALMRDYLGDQWSVANWEGFAAAAKASSSPIARLFFATEEAPQNLKEYDPEWGRAFYEGTVALHCPHDRMLAQVKKPMLLTHHAHHIDPETGDLVGALSDFQAQKVQEIVRSTGVRIDYQSFPDALHMMHLFDPALYTQVLREWAATLPDA

SEQ ID NO: 2 - DNA, 948 bp, Sphingomonas sp.
  source 1..948: mol_type = genomic DNA
atgacgagcgaaaccggcgcgccgcatccggcgcatcgcaacatttttgtgagccatagctttccggaacagcaagtggatctgggcgaagtgaccctgaactatgtggaagcgggcgatgcgggcaaaccggcgctgctgctggtgccggaacagaccggcagctggtggagctatgaaccgagcattgcgatgctggcggaaaactttcatgtgtttgcggtggatatgcgcggccaaggccgcagcgattggaccccgcgccgctatagcctggataactttggcaacgatctggtgcgctttattgcgctggtgattaagcgccctaccatcgtggctggtaacagcagcgggggtgtcttggctgcgtggctgagcgcgtatgcgatgccgggtcagattcgcggcgcgctgtgcgaagatgcgccgttttttgcgagcgaactgaccccggcgtatggccatccgattcgccaagcggcgggcccggcgtttgcgctgatgcgcgattatctgggcgatcagtggagcgtggcgaactgggaaggctttgcggcggcggcgaaagcgagcagcagcccgattgcgcgcctgttttttgcgaccgaagaagcgccgcagaacctgaaagaatatgatccggaatggggccgcgcgttttatgaaggcaccgtggcgctgcattgcccgcatgatcgcatgctggcgcaagtgaaaaaaccgatgctgctgacccatcatgcgcatcatattgatccggaaaccggcgatctggtgggcgcgctgagcgattttcaagcgcagaaagtgcaagaaattgtgcgcagcaccggcgtgcgcattgattatcagagctttccggatgcgctgcacatgatgcatctgtttgatccggcgctgtatacccaagtgctgcgcgaatgggcggcgaccctgccggatgcg

SEQ ID NO: 3 - DNA, 33 bp, synthetic construct
  source 1..33: mol_type = other DNA
gatataccatggggatgacgagcgaaaccggcg

SEQ ID NO: 4 - DNA, 30 bp, synthetic construct
  source 1..30: mol_type = other DNA
cgagtgcggccgccgcatccggcagggtcg

SEQ ID NO: 5 - protein, 344 aa, Sphingomonas sp.
MKLRLTILLAAFAAAPLGAQTVVPSFTLPPSNQLSPQALDVLARMRAATAPDAIKGDLAKQRAFYQKYNDDRLAEMRRNFTTRERRETIGGVMVDSVEPAAGIAPRNAGRVLINVHGGAFMWGSGSGALVEAIPIAATMRVRVVTVDYRLTPEFKYPAASEDVAAVYRALLKRYPAANIGIYGCSAGGVITAQATAWIRRLKLPKPGAIGTFCGTGASYSGDSPYLAGPITGGAALPVPALPATLPTPYMTSIPVTDAAAYPLLSDAEVRAMPPTLLLAGGRDFAVSALTLAHRRLGAAGVPSELYLFDGLPHAFFVWPDMPESTEAYSLIARFFDRYLGHGRK

SEQ ID NO: 6 - DNA, 1032 bp, Sphingomonas sp.
  source 1..1032: mol_type = genomic DNA
atgaagttgcgcctgacgatattgctggcggcgtttgctgctgcgccattaggagcgcaaactgttgtccctagctttacactgccgccctcgaatcaactgagcccccaggccctggatgtgcttgcgcgcatgagagcagctacagctccggacgcgatcaaaggagatcttgccaaacaacgggctttttaccagaaatacaacgacgacagattagcagagatgcgccgcaactttacgacacgggaacggcgtgagaccataggcggagtcatggttgacagtgtagaacctgccgccggaattgcgccgcgcaatgcggggcgtgtgttgataaacgtgcatggtggagctttcatgtgggggtcaggtagcggagccctggtagaagctatacctattgcagccaccatgcgtgtaagagttgtaaccgtagactatcggcttactccggagttcaaataccccgcggcctctgaggacgtggcagcggtgtaccgggctctgttgaagcggtacccggctgcaaacatcggcatctatggatgttctgcaggaggtgtaattacagcgcaagctactgcttggattcgccggttgaagttaccaaagccaggagctatcggaacgttctgtggtactggcgccagctacagtggggactccccatacctggccgggccgattacaggtggagcggcccttcccgtaccagcgttaccagcgacattaccaacaccttatatgacatcaatcccagtaaccgatgcggctgcgtatccccttttaagcgacgccgaggtccgtgccatgcctccgaccctgctgttagccggtgggagagacttcgctgttagtgctttgacacttgcacacagacgccttggggccgccggagttccatccgaactttatttgtttgatggattgccacatgctttctttgtgtggccagacatgccagagtctacagaagcctatagtcttattgctcgtttctttgatcgttatttaggacatggtcgcaaa

SEQ ID NO: 7 - DNA, 38 bp, synthetic construct
  source 1..38: mol_type = other DNA
gatataccatggggatgaagttgcgcctgacgatattg

SEQ ID NO: 8 - DNA, 39 bp, synthetic construct
  source 1..39: mol_type = other DNA
ctcgagtgcggccgctttgcgaccatgtcctaaataacg